European Patent Application EP 4 190 812 A1, published June 7, 2023. Title: ANTI-CD79B ANTIBODY-DRUG CONJUGATE, AND PREPARATION METHOD THEREFOR AND PHARMACEUTICAL USE THEREOF. Applicant: Tuojie Biotech (Shanghai) Co., Ltd. Application PCT/CN2021/108666. The sequence listing filed with the application follows.

SEQUENCE LISTING (33 sequences)

SEQ ID NO: 1 - protein, 433 aa, Artificial Sequence
  Human CD79B ECD-hFc
ARSEDRYRNPKGSACSRIWQSPRFIARKRGFTVKMHCYMNSASGNVSWLWKQEMDENPQQLKLEKGRMEESQNESLATLTIQGIRFEDNGIYFCQQKCNNTSEVYQGCGTELRVMGFSTLAQLKQRNTLKDGIIMIQTLLIILFIIVPIFLLLDKDDSKAGMEEDHTYEGLDIDQTATYEDIVTLRTGEVKWSVGEHPGQEEPKSCDKTHTCPPCPAPELLGGPSVFLFPPKPKDTLMISRTPEVTCVVVDVSHEDPEVKFNWYVDGVEVHNAKTKPREEQYNSTYRVVSVLTVLHQDWLNGKEYKCKVSNKALPAPIEKTISKAKGQPREPQVYTLPPSREEMTKNQVSLTCLVKGFYPSDIAVEWESNGQPENNYKTTPPVLDSDGSFFLYSKLTVDKSRWQQGNVFSCSVMHEALHNHYTQKSLSLSPGK

SEQ ID NO: 2 - protein, 207 aa, Artificial Sequence
  Human CD79B ECD-His
ARSEDRYRNPKGSACSRIWQSPRFIARKRGFTVKMHCYMNSASGNVSWLWKQEMDENPQQLKLEKGRMEESQNESLATLTIQGIRFEDNGIYFCQQKCNNTSEVYQGCGTELRVMGFSTLAQLKQRNTLKDGIIMIQTLLIILFIIVPIFLLLDKDDSKAGMEEDHTYEGLDIDQTATYEDIVTLRTGEVKWSVGEHPGQEHHHHHH

SEQ ID NO: 3 - protein, 117 aa, Mus musculus
QVQLQQSGAELARPGASVKLSCKASGSSFTSYGINWVKQRTGQGLEWIGEIFPRSGNTYYNEKFEGKATLTADKSSSTAYMELRSLTSEDSAVYFCAKGDLGDFDYWGQGTTLTVSS

SEQ ID NO: 4 - protein, 112 aa, Mus musculus
DFLMTQTPLSLPVRLGDQASISCRSSQSIVHSDGNTYFEWYLQKPGQSPKLLIYKVSNRFSGVPDRFSGSGSGTDFTLKISRVEAEDLGVYYCFQGSHVPWTFGGGTKLEIK

SEQ ID NO: 5 - protein, 119 aa, Mus musculus
QVQLQQSGAELARPGASVKLSCKASGYTFTTYGINWVKQRTGQGLEWIGEIYPRSGNIYYNEKFKGKATLTADKSSSTAYMELRSLTSEDSAVYFCARGSDYDGDFAYWGQGTLVTVSA

SEQ ID NO: 6 - protein, 112 aa, Mus musculus
DVLMTQTPLSLPVSLGDQASISCRSSQSIVHHDGNTYLEWYLQKPGQSPKLLIYKVSNRFSGVPDRFSGSGSGTDFTLKISRVEAEDLGVYYCFQGSHVPWTFGGGTQLEIK

SEQ ID NO: 7 - protein, 7 aa, Mus musculus
GSSFTSY

SEQ ID NO: 8 - protein, 6 aa, Mus musculus
FPRSGN

SEQ ID NO: 9 - protein, 8 aa, Mus musculus
GDLGDFDY

SEQ ID NO: 10 - protein, 16 aa, Mus musculus
RSSQSIVHSDGNTYFE

SEQ ID NO: 11 - protein, 7 aa, Mus musculus
KVSNRFS

SEQ ID NO: 12 - protein, 9 aa, Mus musculus
FQGSHVPWT

SEQ ID NO: 13 - protein, 7 aa, Mus musculus
GYTFTTY

SEQ ID NO: 14 - protein, 6 aa, Mus musculus
YPRSGN

SEQ ID NO: 15 - protein, 10 aa, Mus musculus
GSDYDGDFAY

SEQ ID NO: 16 - protein, 16 aa, Mus musculus
RSSQSIVHHDGNTYLE

SEQ ID NO: 17 - protein, 7 aa, Mus musculus
KVSNRFS

SEQ ID NO: 18 - protein, 9 aa, Mus musculus
FQGSHVPWT

SEQ ID NO: 19 - protein, 117 aa, Artificial Sequence
  Heavy chain variable region of hAb015-10 humanized antibody
EVQLVQSGAEVKKPGSSVKVSCKASGSSFSSYGINWVKQAPGQGLEWIGEIFPRSGNTYYNEKFEGRATLTADKSTSTAYMELRSLRSEDTAVYYCAKGDLGDFDYWGQGTTVTVSS

SEQ ID NO: 20 - protein, 112 aa, Artificial Sequence
  Light chain variable region of hAb015-10 humanized antibody
DFVMTQTPLSLPVTPGEPASISCRSSQSIVHSDGNTYFEWYLQKPGQSPKLLIYKVSNRFSGVPDRFSGSGSGTDFTLKISRVEAEDVGVYYCFQGSHVPWTFGGGTKVEIK

SEQ ID NO: 21 - protein, 119 aa, Artificial Sequence
  Heavy chain variable region of hAb017-10 humanized antibody
EVQLVQSGAEVKKPGASVKVSCKASGYTFTTYGINWVKQAPGQGLEWIGEIYPRSGNIYYNEKFKGKATLTADKSTSTAYMELRSLRSDDTAVYYCARGSDYDGDFAYWGQGTLVTVSS

SEQ ID NO: 22 - protein, 112 aa, Artificial Sequence
  Light chain variable region of hAb017-10 humanized antibody
DVVMTQTPLSLPVTPGEPASISCRSSQSIVHHDGNTYLEWYLQKPGQSPQLLIYKVSNRFSGVPDRFSGSGSGTDFTLKISRVEAEDVGVYYCFQGSHVPWTFGGGTKVEIK

SEQ ID NO: 23 - protein, 7 aa, Artificial Sequence
  Mutated HCDR2
GSSFSSY

SEQ ID NO: 24 - protein, 7 aa, Artificial Sequence
  General formula of HCDR1
  VARIANT (2)..(2): Xaa is S or Y
  VARIANT (3)..(3): Xaa is S or T
  VARIANT (5)..(5): Xaa is T or S
  VARIANT (6)..(6): Xaa is S or T
GXXFXXY

SEQ ID NO: 25 - protein, 6 aa, Artificial Sequence
  General formula of HCDR2
  VARIANT (1)..(1): Xaa is F or Y
XPRSGN

SEQ ID NO: 26 - protein, 10 aa, Artificial Sequence
  General formula of HCDR3
  VARIANT (1)..(1): Xaa is absent or G
  VARIANT (2)..(2): Xaa is absent or S
  VARIANT (3)..(3): Xaa is G or D
  VARIANT (4)..(4): Xaa is D or Y
  VARIANT (5)..(5): Xaa is L or D
  VARIANT (9)..(9): Xaa is D or A
XXXXXGDFXY

SEQ ID NO: 27 - protein, 15 aa, Artificial Sequence
  General formula of LCDR1
  VARIANT (9)..(9): Xaa is S or H
  VARIANT (14)..(14): Xaa is F or L
RSSQSIVHXGNTYXE

SEQ ID NO: 28 - protein, 447 aa, Artificial Sequence
  Heavy chain of hAb015-10 humanized antibody
EVQLVQSGAEVKKPGSSVKVSCKASGSSFSSYGINWVKQAPGQGLEWIGEIFPRSGNTYYNEKFEGRATLTADKSTSTAYMELRSLRSEDTAVYYCAKGDLGDFDYWGQGTTVTVSSASTKGPSVFPLAPSSKSTSGGTAALGCLVKDYFPEPVTVSWNSGALTSGVHTFPAVLQSSGLYSLSSVVTVPSSSLGTQTYICNVNHKPSNTKVDKKVEPKSCDKTHTCPPCPAPELLGGPSVFLFPPKPKDTLMISRTPEVTCVVVDVSHEDPEVKFNWYVDGVEVHNAKTKPREEQYNSTYRVVSVLTVLHQDWLNGKEYKCKVSNKALPAPIEKTISKAKGQPREPQVYTLPPSREEMTKNQVSLTCLVKGFYPSDIAVEWESNGQPENNYKTTPPVLDSDGSFFLYSKLTVDKSRWQQGNVFSCSVMHEALHNHYTQKSLSLSPGK

SEQ ID NO: 29 - protein, 219 aa, Artificial Sequence
  Light chain of hAb015-10 humanized antibody
DFVMTQTPLSLPVTPGEPASISCRSSQSIVHSDGNTYFEWYLQKPGQSPKLLIYKVSNRFSGVPDRFSGSGSGTDFTLKISRVEAEDVGVYYCFQGSHVPWTFGGGTKVEIKRTVAAPSVFIFPPSDEQLKSGTASVVCLLNNFYPREAKVQWKVDNALQSGNSQESVTEQDSKDSTYSLSSTLTLSKADYEKHKVYACEVTHQGLSSPVTKSFNRGEC

SEQ ID NO: 30 - protein, 449 aa, Artificial Sequence
  Heavy chain of hAb017-10 humanized antibody
EVQLVQSGAEVKKPGASVKVSCKASGYTFTTYGINWVKQAPGQGLEWIGEIYPRSGNIYYNEKFKGKATLTADKSTSTAYMELRSLRSDDTAVYYCARGSDYDGDFAYWGQGTLVTVSSASTKGPSVFPLAPSSKSTSGGTAALGCLVKDYFPEPVTVSWNSGALTSGVHTFPAVLQSSGLYSLSSVVTVPSSSLGTQTYICNVNHKPSNTKVDKKVEPKSCDKTHTCPPCPAPELLGGPSVFLFPPKPKDTLMISRTPEVTCVVVDVSHEDPEVKFNWYVDGVEVHNAKTKPREEQYNSTYRVVSVLTVLHQDWLNGKEYKCKVSNKALPAPIEKTISKAKGQPREPQVYTLPPSREEMTKNQVSLTCLVKGFYPSDIAVEWESNGQPENNYKTTPPVLDSDGSFFLYSKLTVDKSRWQQGNVFSCSVMHEALHNHYTQKSLSLSPGK

SEQ ID NO: 31 - protein, 219 aa, Artificial Sequence
  Light chain of hAb017-10 humanized antibody
DVVMTQTPLSLPVTPGEPASISCRSSQSIVHHDGNTYLEWYLQKPGQSPQLLIYKVSNRFSGVPDRFSGSGSGTDFTLKISRVEAEDVGVYYCFQGSHVPWTFGGGTKVEIKRTVAAPSVFIFPPSDEQLKSGTASVVCLLNNFYPREAKVQWKVDNALQSGNSQESVTEQDSKDSTYSLSSTLTLSKADYEKHKVYACEVTHQGLSSPVTKSFNRGEC

SEQ ID NO: 32 - protein, 447 aa, Artificial Sequence
  Heavy chain of SN8
EVQLVESGGGLVQPGGSLRLSCAASGYTFSSYWIEWVRQAPGKGLEWIGEILPGGGDTNYNEIFKGRATFSADTSKNTAYLQMNSLRAEDTAVYYCTRRVPIRLDYWGQGTLVTVSSASTKGPSVFPLAPSSKSTSGGTAALGCLVKDYFPEPVTVSWNSGALTSGVHTFPAVLQSSGLYSLSSVVTVPSSSLGTQTYICNVNHKPSNTKVDKKVEPKSCDKTHTCPPCPAPELLGGPSVFLFPPKPKDTLMISRTPEVTCVVVDVSHEDPEVKFNWYVDGVEVHNAKTKPREEQYNSTYRVVSVLTVLHQDWLNGKEYKCKVSNKALPAPIEKTISKAKGQPREPQVYTLPPSREEMTKNQVSLTCLVKGFYPSDIAVEWESNGQPENNYKTTPPVLDSDGSFFLYSKLTVDKSRWQQGNVFSCSVMHEALHNHYTQKSLSLSPGK

SEQ ID NO: 33 - protein, 218 aa, Artificial Sequence
  Light chain of SN8
DIQLTQSPSSLSASVGDRVTITCKASQSVDYEGDSFLNWYQQKPGKAPKLLIYAASNLESGVPSRFSGSGSGTDFTLTISSLQPEDFATYYCQQSNEDPLTFGQGTKVEIKRTVAAPSVFIFPPSDEQLKSGTASVVCLLNNFYPREAKVQWKVDNALQSGNSQESVTEQDSKDSTYSLSSTLTLSKADYEKHKVYACEVTHQGLSSPVTKSFNRGEC